European Patent Application EP 4 487 875 A1, published January 8, 2025. Title: Medicine for diseases caused by frameshift mutation. Applicant: JCR Pharmaceuticals Co., Ltd. Application JP. The sequence listing filed with the application follows.

SEQUENCE LISTING (111 sequences)

SEQ ID NO: 1 - DNA, 25 bp, synthetic construct
  misc_feature 1..25: note = Forward primer used in Example 1
  source 1..25: mol_type = other DNA
tgaagtcaaatcagaattcatcaag

SEQ ID NO: 2 - DNA, 22 bp, synthetic construct
  misc_feature 1..22: note = Reverse primer used in Example 1
  source 1..22: mol_type = other DNA
atcagtggcattcacagaagtg

SEQ ID NO: 3 - DNA, 16 bp, synthetic construct
  misc_feature 1..16: note = Barcode sequence used in Example 1
  source 1..16: mol_type = other DNA
cgctcttccgatctcg

SEQ ID NO: 4 - DNA, 15 bp, synthetic construct
  misc_feature 1..15: note = Barcode sequence used in Example 1
  source 1..15: mol_type = other DNA
cgcttccgatctgac

SEQ ID NO: 5 - DNA, 18 bp, synthetic construct
  misc_feature 1..18: note = Forward primer used in Example 1
  source 1..18: mol_type = other DNA
aactcatcagctgcaccg

SEQ ID NO: 6 - DNA, 21 bp, synthetic construct
  misc_feature 1..21: note = Reverse primer used in Example 1
  source 1..21: mol_type = other DNA
gggctagcaatcatgcacttc

SEQ ID NO: 7 - DNA, 20 bp, synthetic construct
  misc_feature 1..20: note = EYS-specific primer
  source 1..20: mol_type = other DNA
gttggccagtgtcatgcttc

SEQ ID NO: 8 - DNA, 20 bp, synthetic construct
  misc_feature 1..20: note = EYS-specific primer
  source 1..20: mol_type = other DNA
cgccaaggttgtagcgaagt

SEQ ID NO: 9 - DNA, 20 bp, synthetic construct
  misc_feature 1..20: note = GAPDH-specific primer
  source 1..20: mol_type = other DNA
tgaccacagtccatgccatc

SEQ ID NO: 10 - DNA, 21 bp, synthetic construct
  misc_feature 1..21: note = GAPDH-specific primer
  source 1..21: mol_type = other DNA
ttactccttggaggccatgtg

SEQ ID NO: 11 - DNA, 33 bp, synthetic construct
  misc_feature 1..33: note = Sequence shown in Figure 1
  source 1..33: mol_type = other DNA
tccattaccctatcaaagtaatttggatgttaa

SEQ ID NO: 12 - DNA, 33 bp, synthetic construct
  misc_feature 1..33: note = Sequence shown in Figure 1
  source 1..33: mol_type = other DNA
ttaacatccaaattactttgatagggtaatgga

SEQ ID NO: 13 - DNA, 33 bp, synthetic construct
  misc_feature 1..33: note = Sequence shown in Figure 1
  source 1..33: mol_type = other DNA
tccattaccctatcaagtaatttggatgttaat

SEQ ID NO: 14 - DNA, 33 bp, synthetic construct
  misc_feature 1..33: note = Sequence shown in Figure 1
  source 1..33: mol_type = other DNA
attaacatccaaattacttgatagggtaatgga

SEQ ID NO: 15 - DNA, 40 bp, synthetic construct
  misc_feature 1..40: note = Sequence shown in Figure 2
  source 1..40: mol_type = other DNA
aattaacatccaaattactttgatagggtaatggattctt

SEQ ID NO: 16 - DNA, 39 bp, synthetic construct
  misc_feature 1..39: note = Sequence shown in Figure 2
  source 1..39: mol_type = other DNA
aattaacatccaaattacttgatagggtaatggattctt

SEQ ID NO: 17 - DNA, 39 bp, synthetic construct
  misc_feature 1..39: note = Sequence shown in Figure 2
  source 1..39: mol_type = other DNA
aatgaacatccaaattacttgatagggtaatggattctt

SEQ ID NO: 18 - DNA, 39 bp, synthetic construct
  misc_feature 1..39: note = Sequence shown in Figure 2
  source 1..39: mol_type = other DNA
aattaacagccaaattacttgatagggtaatggattctt

SEQ ID NO: 19 - DNA, 39 bp, synthetic construct
  misc_feature 1..39: note = Sequence shown in Figure 2
  source 1..39: mol_type = other DNA
aattaacatccaaattacttgatagggtaatggactctt

SEQ ID NO: 20 - DNA, 39 bp, synthetic construct
  misc_feature 1..39: note = Sequence shown in Figure 2
  source 1..39: mol_type = other DNA
aattaacatccaaattacttgatagggtaatggatcctt

SEQ ID NO: 21 - DNA, 39 bp, synthetic construct
  misc_feature 1..39: note = Sequence shown in Figure 2
  source 1..39: mol_type = other DNA
aattaacatccaaattacttgatagggtaatggattcct

SEQ ID NO: 22 - DNA, 39 bp, synthetic construct
  misc_feature 1..39: note = Sequence shown in Figure 2
  source 1..39: mol_type = other DNA
aattagcatccaaattacttgatagggtaatggattctt

SEQ ID NO: 23 - DNA, 39 bp, synthetic construct
  misc_feature 1..39: note = Sequence shown in Figure 2
  source 1..39: mol_type = other DNA
aataacatccaaattacttttgatagggtattgattctt

SEQ ID NO: 24 - DNA, 40 bp, synthetic construct
  misc_feature 1..40: note = Sequence shown in Figure 2
  source 1..40: mol_type = other DNA
attaacatccaaattacttttgttagggtaatgaattttt

SEQ ID NO: 25 - DNA, 61 bp, synthetic construct
  misc_feature 1..61: note = Sequence shown in Figure 4
  source 1..61: mol_type = other DNA
atggattggggcacgctgcagacgatcctgggggggtgtgaacaaacactccaccagcatt

SEQ ID NO: 26 - DNA, 61 bp, synthetic construct
  misc_feature 1..61: note = Sequence shown in Figure 4
  source 1..61: mol_type = other DNA
aatgctggtggagtgtttgttcacacccccccaggatcgtctgcagcgtgccccaatccat

SEQ ID NO: 27 - DNA, 61 bp, synthetic construct
  misc_feature 1..61: note = Sequence shown in Figure 4
  source 1..61: mol_type = other DNA
tcccacatccggctatgggccctgcaagctgatcttcgtgtccacgccagcgctcctagtg

SEQ ID NO: 28 - DNA, 61 bp, synthetic construct
  misc_feature 1..61: note = Sequence shown in Figure 4
  source 1..61: mol_type = other DNA
cactaggagcgctggcgtggacacgaagatcagcttgcagggcccatagccggatgtggga

SEQ ID NO: 29 - DNA, 61 bp, synthetic construct
  misc_feature 1..61: note = Sequence shown in Figure 6
  source 1..61: mol_type = other DNA
ccgccgccgcccccggcaccgcagccccccccagacgcggggcgccccggccgccgacgac

SEQ ID NO: 30 - DNA, 61 bp, synthetic construct
  misc_feature 1..61: note = Sequence shown in Figure 6
  source 1..61: mol_type = other DNA
gtcgtcggcggccggggcgccccgcgtctggggggggctgcggtgccgggggcggcggcgg

SEQ ID NO: 31 - DNA, 61 bp, synthetic construct
  misc_feature 1..61: note = Sequence shown in Figure 6
  source 1..61: mol_type = other DNA
agaaggagaagggcgccggcgccggggggggaggagaagaagggggcgggcgagggcggca

SEQ ID NO: 32 - DNA, 61 bp, synthetic construct
  misc_feature 1..61: note = Sequence shown in Figure 6
  source 1..61: mol_type = other DNA
tgccgccctcgcccgcccccttcttctcctccccccccggcgccggcgcccttctccttct

SEQ ID NO: 33 - DNA, 61 bp, synthetic construct
  misc_feature 1..61: note = Sequence shown in Figure 7
  source 1..61: mol_type = other DNA
cttagaagatactttatttccttcctcaaaagaagctcaagaaagacaaccaagagagctc

SEQ ID NO: 34 - DNA, 61 bp, synthetic construct
  misc_feature 1..61: note = Sequence shown in Figure 7
  source 1..61: mol_type = other DNA
gagctctcttggttgtctttcttgagcttcttttgaggaaggaaataaagtatcttctaag

SEQ ID NO: 35 - DNA, 61 bp, synthetic construct
  misc_feature 1..61: note = Sequence shown in Figure 8
  source 1..61: mol_type = other DNA
ctgagcatgttcactggctacctgtccaacaaaccgcttctatccaccgccgcccaagggc

SEQ ID NO: 36 - DNA, 61 bp, synthetic construct
  misc_feature 1..61: note = Sequence shown in Figure 8
  source 1..61: mol_type = other DNA
gcccttgggcggcggtggatagaagcggtttgttggacaggtagccagtgaacatgctcag

SEQ ID NO: 37 - DNA, 61 bp, synthetic construct
  misc_feature 1..61: note = Sequence shown in Figure 9
  source 1..61: mol_type = other DNA
gtctgctgatcatcgaagctccccaggtcccctccttactcaacatttggagagagcagtt

SEQ ID NO: 38 - DNA, 61 bp, synthetic construct
  misc_feature 1..61: note = Sequence shown in Figure 9
  source 1..61: mol_type = other DNA
aactgctctctccaaatgttgagtaaggaggggacctggggagcttcgatgatcagcagac

SEQ ID NO: 39 - DNA, 61 bp, synthetic construct
  misc_feature 1..61: note = Sequence shown in Figure 10
  source 1..61: mol_type = other DNA
ccaaaacccctaaacctggagaacttggggggaagaatatctgggtcagtggcttggagag

SEQ ID NO: 40 - DNA, 61 bp, synthetic construct
  misc_feature 1..61: note = Sequence shown in Figure 10
  source 1..61: mol_type = other DNA
ctctccaagccactgacccagatattcttccccccaagttctccaggtttaggggttttgg

SEQ ID NO: 41 - DNA, 22 bp, synthetic construct
  source 1..22: mol_type = other DNA
acctgtagacccatttcacctc

SEQ ID NO: 42 - DNA, 19 bp, synthetic construct
  source 1..19: mol_type = other DNA
cacacaggagaggtcggtg

SEQ ID NO: 43 - DNA, 22 bp, synthetic construct
  source 1..22: mol_type = other DNA
ctcgtacttgccgttcttcttc

SEQ ID NO: 44 - DNA, 22 bp, synthetic construct
  source 1..22: mol_type = other DNA
cttcctgctcaaggccatcatg

SEQ ID NO: 45 - DNA, 22 bp, synthetic construct
  source 1..22: mol_type = other DNA
cagaggcaactgtttttgtcag

SEQ ID NO: 46 - DNA, 23 bp, synthetic construct
  source 1..23: mol_type = other DNA
agacctgaagctggtcatcaatg

SEQ ID NO: 47 - DNA, 19 bp, synthetic construct
  source 1..19: mol_type = other DNA
ccctggacggggctaaagc

SEQ ID NO: 48 - DNA, 21 bp, synthetic construct
  source 1..21: mol_type = other DNA
ccccagattgggatgtctctg

SEQ ID NO: 49 - DNA, 15 bp, synthetic construct
  source 1..15: mol_type = other DNA
cgcttccgatctctg

SEQ ID NO: 50 - DNA, 15 bp, synthetic construct
  source 1..15: mol_type = other DNA
cgcttccgatctgac

SEQ ID NO: 51 - DNA, 40 bp, synthetic construct
  source 1..40: mol_type = other DNA
ctaaacctggagaacttggggggaagaatatctgggtcag

SEQ ID NO: 52 - DNA, 39 bp, synthetic construct
  source 1..39: mol_type = other DNA
ctaaacctggagaacttgggggaagaatatctgggtcag

SEQ ID NO: 53 - DNA, 39 bp, synthetic construct
  source 1..39: mol_type = other DNA
ctaaacctggaggacttgggggaagaatatctgggtcag

SEQ ID NO: 54 - DNA, 39 bp, synthetic construct
  source 1..39: mol_type = other DNA
ctaaacctggagcacttgggggaagaatatctgggtcag

SEQ ID NO: 55 - DNA, 38 bp, synthetic construct
  source 1..38: mol_type = other DNA
ctaaacctggagaacttggggaagaatatctgggtcag

SEQ ID NO: 56 - DNA, 39 bp, synthetic construct
  source 1..39: mol_type = other DNA
ctaaacctggagagcttgggggaagaatatctgggtcag

SEQ ID NO: 57 - DNA, 39 bp, synthetic construct
  source 1..39: mol_type = other DNA
ctaaaactggagaacttgggggaagaatatctgggtcag

SEQ ID NO: 58 - DNA, 39 bp, synthetic construct
  source 1..39: mol_type = other DNA
ctaaacctggggaacttgggggaagaatatctgggtcag

SEQ ID NO: 59 - DNA, 61 bp, synthetic construct
  source 1..61: mol_type = other DNA
accaggtggaatatgatcagctgacccccccggcgctccaggtgcagaggaagccaccagg

SEQ ID NO: 60 - DNA, 61 bp, synthetic construct
  source 1..61: mol_type = other DNA
cctggtggcttcctctgcacctggagcgccgggggggtcagctgatcatattccacctggt

SEQ ID NO: 61 - DNA, 40 bp, synthetic construct
  source 1..40: mol_type = other DNA
cctctgcacctggagcgccgggggggtcagctgatcatat

SEQ ID NO: 62 - DNA, 39 bp, synthetic construct
  source 1..39: mol_type = other DNA
cctctgcacctggagcgccggggggtcagctgatcatat

SEQ ID NO: 63 - DNA, 40 bp, synthetic construct
  source 1..40: mol_type = other DNA
ctctgcacctggagcgccggggggggtcagctgatcatat

SEQ ID NO: 64 - DNA, 40 bp, synthetic construct
  source 1..40: mol_type = other DNA
ctccgcacctggagcgccggggggggtcagctgatcatat

SEQ ID NO: 65 - DNA, 38 bp, synthetic construct
  source 1..38: mol_type = other DNA
cctctgcacctggagcgccgggggtcagctgatcatat

SEQ ID NO: 66 - DNA, 40 bp, synthetic construct
  source 1..40: mol_type = other DNA
ctctgcccctggagcgccggggggggtcagctgatcatat

SEQ ID NO: 67 - DNA, 39 bp, synthetic construct
  source 1..39: mol_type = other DNA
cctctgcccctggagcgccggggggtcagctgatcatat

SEQ ID NO: 68 - DNA, 39 bp, synthetic construct
  source 1..39: mol_type = other DNA
cctctgcacctggagcgcccgggggtcagctgatcatat

SEQ ID NO: 69 - DNA, 39 bp, synthetic construct
  source 1..39: mol_type = other DNA
cctctgcacctggagcgccggggggtcagctgatcatac

SEQ ID NO: 70 - DNA, 39 bp, synthetic construct
  source 1..39: mol_type = other DNA
cctctgcacctggagcgccggtgggtcagctgatcatat

SEQ ID NO: 71 - DNA, 40 bp, synthetic construct
  source 1..40: mol_type = other DNA
ccgcccccttcttctcctccccccccggcgccggcgccct

SEQ ID NO: 72 - DNA, 39 bp, synthetic construct
  source 1..39: mol_type = other DNA
ccgcccccttcttctcctcccccccggcgccggcgccct

SEQ ID NO: 73 - DNA, 38 bp, synthetic construct
  source 1..38: mol_type = other DNA
ccgcccccttcttctcctccccccggcgccggcgccct

SEQ ID NO: 74 - DNA, 39 bp, synthetic construct
  source 1..39: mol_type = other DNA
ccgcccccttcttcccctcccccccggcgccggcgccct

SEQ ID NO: 75 - DNA, 39 bp, synthetic construct
  source 1..39: mol_type = other DNA
ccgcccccttcttcgcctcccccccggcgccggcgccct

SEQ ID NO: 76 - DNA, 39 bp, synthetic construct
  source 1..39: mol_type = other DNA
ccgcccccttcttctccgcccccccggcgccggcgccct

SEQ ID NO: 77 - DNA, 39 bp, synthetic construct
  source 1..39: mol_type = other DNA
ccgcccccttcgtctcctcccccccggcgccggcgccct

SEQ ID NO: 78 - DNA, 39 bp, synthetic construct
  source 1..39: mol_type = other DNA
ccgcccccttctcctcctcccccccggcgccggcgccct

SEQ ID NO: 79 - DNA, 39 bp, synthetic construct
  source 1..39: mol_type = other DNA
ccgcccccttctgctcctcccccccggcgccggcgccct

SEQ ID NO: 80 - DNA, 40 bp, synthetic construct
  source 1..40: mol_type = other DNA
gtcatggtgaccgggatggccatcaaagtaggaggaatgt

SEQ ID NO: 81 - DNA, 39 bp, synthetic construct
  source 1..39: mol_type = other DNA
gtcatggtcacagggatggcgtcgaagtaggacgagtga

SEQ ID NO: 82 - DNA, 39 bp, synthetic construct
  source 1..39: mol_type = other DNA
gtcatggtcacagggatggcgtcaaagtaggacgagtga

SEQ ID NO: 83 - DNA, 39 bp, synthetic construct
  source 1..39: mol_type = other DNA
gtcatggtcacagggatggcgtcgcagtaggacgagtga

SEQ ID NO: 84 - DNA, 34 bp, synthetic construct
  source 1..34: mol_type = other DNA
ggtcacagggatggcgtcgaagtaggacgagtga

SEQ ID NO: 85 - DNA, 14 bp, synthetic construct
  source 1..14: mol_type = other DNA
gtcatggtcacagg

SEQ ID NO: 86 - DNA, 39 bp, synthetic construct
  source 1..39: mol_type = other DNA
gtcatggtcacagggatggcgtcgaagtaggacgaccga

SEQ ID NO: 87 - DNA, 39 bp, synthetic construct
  source 1..39: mol_type = other DNA
gtcatggtcacagggatggcgtcgaagtaggacgtgtga

SEQ ID NO: 88 - DNA, 39 bp, synthetic construct
  source 1..39: mol_type = other DNA
gtcatggtcacggggatggcgtcgaagtaggacgagtga

SEQ ID NO: 89 - DNA, 14 bp, synthetic construct
  source 1..14: mol_type = other DNA
gtcatggtgaccgg

SEQ ID NO: 90 - DNA, 39 bp, synthetic construct
  source 1..39: mol_type = other DNA
gtcatggtgaccgggatggcgtcgaagtaggacgagtga

SEQ ID NO: 91 - DNA, 39 bp, synthetic construct
  source 1..39: mol_type = other DNA
gtcatggttacagggatggcgtcaaagtaggacgagtga

SEQ ID NO: 92 - DNA, 39 bp, synthetic construct
  source 1..39: mol_type = other DNA
gtcatggttacagggatggcgtcgaagtaggacgagtga

SEQ ID NO: 93 - DNA, 39 bp, synthetic construct
  source 1..39: mol_type = other DNA
gtcctggtccccgggatggcgtcggggtgggacgagtga

SEQ ID NO: 94 - DNA, 60 bp, synthetic construct
  source 1..60: mol_type = other DNA
agagcgattcttcgacctctgcagccccccctcagggggctcgggggacccctgcgcagc

SEQ ID NO: 95 - DNA, 60 bp, synthetic construct
  source 1..60: mol_type = other DNA
gctgcgcaggggtcccccgagccccctgagggggggctgcagaggtcgaagaatcgctct

SEQ ID NO: 96 - DNA, 60 bp, synthetic construct
  source 1..60: mol_type = other DNA
cggcgcacgcgccctacctgatgttcccccccgccgcccttcgggctgcccatcgcgtcg

SEQ ID NO: 97 - DNA, 60 bp, synthetic construct
  source 1..60: mol_type = other DNA
cgacgcgatgggcagcccgaagggcggcgggggggaacatcaggtagggcgcgtgcgccg

SEQ ID NO: 98 - DNA, 60 bp, synthetic construct
  source 1..60: mol_type = other DNA
agagtccttgtgctccgcggccacccccaaaggtcactcaggccctgaacgtcctgacca

SEQ ID NO: 99 - DNA, 60 bp, synthetic construct
  source 1..60: mol_type = other DNA
tggtcaggacgttcagggcctgagtgacctttgggggtggccgcggagcacaaggactct

SEQ ID NO: 100 - DNA, 60 bp, synthetic construct
  source 1..60: mol_type = other DNA
agttctgtgaccaagcatgcaatgtcttgtctgtgggtttgatgctggcgactgtgggca

SEQ ID NO: 101 - DNA, 60 bp, synthetic construct
  source 1..60: mol_type = other DNA
tgcccacagtcgccagcatcaaacccacagacaagacattgcatgcttggtcacagaact

SEQ ID NO: 102 - DNA, 60 bp, synthetic construct
  source 1..60: mol_type = other DNA
ggcagcatcctctacagcttgctcactagccaaagcaaacgcacgtggctccggcagcgc

SEQ ID NO: 103 - DNA, 60 bp, synthetic construct
  source 1..60: mol_type = other DNA
gcgctgccggagccacgtgcgtttgctttggctagtgagcaagctgtagaggatgctgcc

SEQ ID NO: 104 - DNA, 60 bp, synthetic construct
  source 1..60: mol_type = other DNA
ctggtctccatcctttccacccacagaatggacagggtagccacccagctggttgtgagc

SEQ ID NO: 105 - DNA, 60 bp, synthetic construct
  source 1..60: mol_type = other DNA
gctcacaaccagctgggtggctaccctgtccattctgtgggtggaaaggatggagaccag

SEQ ID NO: 106 - DNA, 60 bp, synthetic construct
  source 1..60: mol_type = other DNA
ggactgtggaccaccagctcctgtgggggggaggccctgctcatcaccccagtgctccag

SEQ ID NO: 107 - DNA, 60 bp, synthetic construct
  source 1..60: mol_type = other DNA
ctggagcactggggtgatgagcagggcctcccccccacaggagctggtggtccacagtcc

SEQ ID NO: 108 - DNA, 60 bp, synthetic construct
  source 1..60: mol_type = other DNA
cattgactttcttctgcagattacctgttttcgtgagtctcttggggttagacattaaac

SEQ ID NO: 109 - DNA, 60 bp, synthetic construct
  source 1..60: mol_type = other DNA
gtttaatgtctaaccccaagagactcacgaaaacaggtaatctgcagaagaaagtcaatg

SEQ ID NO: 110 - DNA, 59 bp, synthetic construct
  source 1..59: mol_type = other DNA
aattctgcaatcctcactctgggcagtgtagtgcaaaaaagaagccaaaggacttcagt

SEQ ID NO: 111 - DNA, 59 bp, synthetic construct
  source 1..59: mol_type = other DNA
actgaagtcctttggcttcttttttgcactacactgcccagagtgaggattgcagaatt